European Patent Application EP 4 516 917 A1, published March 5, 2025. Title: Biocatalytic isomerization of a carbohydrate. Applicant: CASCAT GmbH. The sequence listing filed with the application follows.

SEQUENCE LISTING (54 sequences)

SEQ ID NO: 1 - protein, 220 aa, Escherichia coli
MELYLDTSDVVAVKALSRIFPLAGVTTNPSIIAAGKKPLDVVLPQLHEAMGGQGRLFAQVMATTAEGMVNDALKLRSIIADIVVKVPVTAEGLAAIKMLKAEGIPTLGTAVYGAAQGLLSALAGAEYVSPYVNRIDAQGGSGIQTVTDLHQLLKMHAPQAKVLAASFKTPRQALDCLLAGCESITLPLDVAQQMISYPAVDAAVAKFEQDWQGAFGRTSI

SEQ ID NO: 2 - DNA, 663 bp, Escherichia coli
  source 1..663: mol_type = other DNA
atggaactgtatctggatacttcagacgttgttgcggtgaaggcgctgtcacgtatttttccgctggcgggtgtgaccactaacccaagcattatcgccgcgggtaaaaaaccgctggatgttgtgcttccgcaacttcatgaagcgatgggcggtcaggggcgtctgtttgcccaggtaatggctaccactgccgaagggatggttaatgacgcgcttaagctgcgttctattattgcggatatcgtggtgaaagttccggtgaccgccgaggggctggcagctattaagatgttaaaagcggaagggattccgacgctgggaaccgcggtatatggcgcagcacaagggctgctgtcggcgctggcaggtgcggaatatgttagcccttacgttaatcgtattgatgctcagggcggtagcggcattcagactgtgaccgacttacaccagttattgaaaatgcatgcgccgcaggcgaaagtgctggcagcgagtttcaaaaccccgcgtcaggcgctggactgcttactggcaggatgtgaatcaattactctgccactggatgtggcacaacagatgattagctatccggcggttgatgccgctgtggcgaagtttgagcaggactggcagggagcgtttggcagaacgtcgatttaa

SEQ ID NO: 3 - protein, 183 aa, Escherichia coli
MTDKLTSLRQYTTVVADTGDIAAMKLYQPQDATTNPSLILNAAQIPEYRKLIDDAVAWAKQQSNDRAQQIVDATDKLAVNIGLEILKLVPGRISTEVDARLSYDTEASIAKAKRLIKLYNDAGISNDRILIKLASTWQGIRAAEQLEKEGINCNLTLLFSFAQARACAEAGVFLISPYVGEYS

SEQ ID NO: 4 - DNA, 955 bp, Escherichia coli
  source 1..955: mol_type = other DNA
atgacggacaaattgacctcccttcgtcagtacaccaccgtagtggccgacactggggacatcgcggcaatgaagctgtatcaaccgcaggatgccacaaccaacccttctctcattcttaacgcagcgcagattccggaataccgtaagttgattgatgatgctgtcgcctgggcgaaacagcagagcaacgatcgcgcgcagcagatcgtggacgcgaccgacaaactggcagtaaatattggtctggaaatcctgaaactggttccgggccgtatctcaactgaagttgatgcgcgtctttcctatgacaccgaagcgtcaattgcgaaagcaaaacgcctgatcaaactctacaacgatgctggtattagcaacgatcgtattctgatcaaactggcttctacctggcagggtatccgtgctgcagaacagctggaaaaagaaggcatcaactgtaacctgaccctgctgttctccttcgctcaggctcgtgcttgtgcggaagcgggcgtgttcctgatctcgccgtatgttggcgaatattcttgactggtacaaagcgaataccgataagaaagagtacgctccggcagaagatccgggcgtggtttctgtatctgaaatctaccagtactacaaagagcacggttatgaaaccgtggttatgggcgcaagcttccgtaacatcggcgaaattctggaactggcaggctgcgaccgtctgaccatcgcaccggcactgctgaaagagctggcggagagcgaaggggctatcgaacgtaaactgtcttacaccggcgaagtgaaagcgcgtccggcgcgtatcactgagtccgagttcctgtggcagcacaaccaggatccaatggcagtagataaactggcggaaggtatccgtaagtttgctattgaccaggaaaaactggaaaaaatgatcggcgatctgctgtaa

SEQ ID NO: 5 - protein, 258 aa, Escherichia coli
MLRFSANLSMLFGEYDFLARFEKAAQCGFRGVEFMFPYDYDIEELKHVLASNKLEHTLHNLPAGDWAAGERGIACIPGREEEFRDGVAAAIRYARALGNKKINCLVGKTPAGFSSEQIHATLVENLRYAANMLMKEDILLLIEPINHFDIPGFHLTGTRQALKLIDDVGCCNLKIQYDIYHMQRMEGELTNTMTQWADKIGHLQIADNPHRGEPGTGEINYDYLFKVIENSDYNGWVGCEYKPQTTTEAGLRWMDPYR

SEQ ID NO: 6 - DNA, 774 bp, Escherichia coli
  source 1..774: mol_type = genomic DNA
atgttacgtttctctgctaatttatcgatgttatttggagaatatgattttctcgcccgttttgagaaagctgcgcagtgtggttttcgcggcgttgaatttatgtttccttatgactacgacattgaagaattaaaacatgtgctggcgagtaataaactcgaacatacgctgcacaatttaccggcgggtgactgggcggcgggggagcgcggtattgcctgtattcctggccgtgaagaagagtttcgggatggcgtagcagcagcgattcgttatgcccgtgcgctgggtaataaaaaaattaactgtctggtcggtaaaacgccggctggtttcagcagtgaacagattcacgcaacgcttgtagaaaacctgcgttatgccgcgaatatgctgatgaaagaagatattttattactgattgaacctattaaccattttgatattcctggtttccatctcaccggaactcggcaggcgctgaaattgattgatgatgttggttgctgcaatttgaaaattcagtatgacatttatcatatgcagcggatggaaggtgaattaaccaacaccatgactcagtgggctgataaaattggtcacctgcaaattgccgataatccgcatcgcggcgaaccgggaaccggagaaattaattatgattatctctttaaggtaatcgaaaattctgactacaacggttgggttgggtgtgaatataaaccccaaaccaccacggaagccggtttacgctggatggatccgtaccgt

SEQ ID NO: 7 - protein, 396 aa, Arthrobacter sp. FB24
MTLQPTPADRFTFGLWTVGWTGADPFGVATRPALDPVEAVHKLSELGAYGITFHDNDLVPFDATASERELILKNFKAALAETGLKTPMVTTNLFSHPVFKDGGFTSNDRSVRRFALSKVLQNIDLAAELGAETFVMWGGREGSEYDGSKDLSAALDRMKEGVDTAAAYIKDKGYGLRIALEPKPNEPRGDIFLPTVGHGLAFIAQLEHGDIVGLNPETGHEQMAGLNFTHGIAQALWAGKLFHIDLNGQRGIKYDQDLVFGHGDLTSAFFTVDLLENGFPNGGPKYDGPRHFDYKPSRTDGYDGVWESAKSNMSMYLLLKERALAFRADPDVQEALKTSGVFELGEPTLAAGETTADLLADASAFAEFDADAAAQRSFAFVRLNQLAIEHLLGARF

SEQ ID NO: 8 - DNA, 1188 bp, Arthrobacter sp. FB24
  source 1..1188: mol_type = other DNA
atgaccctgcaaccgaccccggcggaccgttttacgtttggcctgtggaccgttggttggaccggcgcagacccgtttggcgtggcgacgcgtccggcactggatccggtggaagctgttcataaactgtctgaactgggcgcgtacggtattaccttccacgataatgacctggtgccgtttgatgcaacggctagtgaacgcgaactgatcctgaaaaactttaaagcggccctggccgaaaccggtctgaaaacgccgatggttaccacgaacctgttttcccatccggtcttcaaagatggcggttttaccagcaatgaccgttcagtccgtcgcttcgccctgtcaaaagtgctgcagaacattgatctggcagctgaactgggcgcagaaacgtttgtgatgtggggcggtcgtgaaggctccgaatatgatggttcgaaagacctgagcgcggccctggatcgcatgaaagaaggtgttgacaccgcagctgcgtatattaaagataaaggctacggtctgcgtatcgcgctggaaccgaaaccgaatgaaccgcgcggcgatattttcctgccgaccgttggccatggtctggcgtttattgcccagctggaacacggcgatatcgtcggtctgaacccggaaaccggccatgaacagatggcaggtctgaattttacccatggtattgcccaagcactgtgggctggtaaactgtttcatattgatctgaacggccagcgtggtatcaaatacgatcaagacctggtctttggccacggtgatctgacctctgcgtttttcacggtggacctgctggaaaacggtttcccgaatggcggtccgaaatatgatggcccgcgtcactttgactacaaaccgtcacgcaccgatggctatgacggtgtttgggaaagcgccaaatctaatatgagtatgtatctgctgctgaaagaacgtgcactggcttttcgtgccgatccggatgtgcaggaagccctgaaaacctcgggcgtttttgaactgggtgaaccgaccctggcggcaggtgaaaccaccgcagatctgctggccgatgcaagcgcatttgctgaattcgatgcggacgctgcggcccaacgctcgtttgcatttgtccgtctgaatcaactggctatcgaacacctgctgggcgcacgcttt

SEQ ID NO: 9 - protein, 575 aa, Paralcaligenes ureilyticus DSM 24591
MSDKEKPVRRSQAWFGRLDRDGFIYRSWMKNRGIPHDQFDGRPVIGICNTFSELTPCNSHFRTLAEQVKIGVWESGGFPLEFPVMSLGETMLRPTAMLFRNLASMDVEESIRGNPLDGVVLLMGCDKTTPSLMMGAASCDLPTIGVSGGPMLSGKFRGRELGSGTDVWKMSEEVRAGQMSQEEFFEAESCMHRSHGHCMTMGTASTMASMVEALGMSLPGNAAIPAVDARRNLLARASGRRIVQMVKDDLVMSKILTRQAFENAIRVNAAIGGSTNAVIHLLAIAGRIGVDLTLADWDALGHKLPCLVDLQPSGTHLMEDFYYAGGVPAVIRELGDVIARDALTVNGQTLWDNCKDAPNWNREVIHAFNEPFKTEAGIAVLRGNLCPDGAVIKPSAATPALLKHKGRAVVFENSEHMHERMDDENLDVDENCVLVLKNCGPRGYPGMAEAGNMPLPPKILRKGITDMVRVSDARMSGTAYGTVVLHVAPEAAAGGPLALVQDGDIIELDVAARKLHLHVSDEELARRREAWQAPPAPMARGWVKLYVEHVQQANLGADLDFLRGKSGAGIPKDNH

SEQ ID NO: 10 - DNA, 1728 bp, Paralcaligenes ureilyticus DSM 24591
  source 1..1728: mol_type = genomic DNA
atgagtgacaaagaaaagcctgtgcgtcgcagccaggcctggttcggacggcttgaccgcgacggtttcatctaccgttcgtggatgaagaatcgaggcatcccgcacgatcagttcgacggtcgcccggtgattggcatttgcaatactttctctgaactgacgccgtgcaattcgcatttccgcaccttggccgagcaggtcaagatcggggtttgggagtcgggcggcttccctctcgagtttccggtcatgtcgctgggcgagacgatgttgcggcctacggccatgctgtttcgcaacctggccagcatggacgtcgaggaatcgatacgcggcaatccgttggatggcgtcgtattgctgatgggctgcgacaaaacgacgccttcgctcatgatgggggcggcgtcctgcgacctgcccactatcggtgtgtcgggcggtcccatgcttagcggcaagtttcgaggccgcgaactgggttcaggcaccgacgtctggaagatgtctgaagaagttcgcgccgggcaaatgtcgcaggaagaatttttcgaagcggaaagctgcatgcatcgctcgcatgggcattgcatgacgatgggtacggcatccacgatggccagcatggtggaagcgctgggcatgagcctgcctggcaacgcggcgattcccgccgtggatgcgcgccgcaatctgctcgcgcgcgcttcgggccggcgcattgtgcagatggtcaaagatgatctggtcatgtcgaaaatcctgacgcgccaggcctttgaaaacgccatccgcgtgaacgccgctatcggtggctcgaccaacgcggtgattcatctgttggcgattgcggggcgtatcggggttgacctgacgcttgccgactgggatgcgctcggccacaaattgccgtgcctggttgatctgcagccttcgggcactcatctgatggaagacttttattatgcgggcggcgtgcccgccgtgatccgcgagctgggcgatgtcattgcccgcgatgccctgacggtgaatggccagaccctgtgggataactgcaaggatgcgccaaactggaatcgcgaggtcatccatgcctttaacgagcctttcaagaccgaggcggggatagccgtactgcgtggcaacctatgccccgatggggccgtcatcaaaccttcggccgccacgccggccctgctcaagcacaagggccgcgcggtcgtgttcgaaaacagcgaacatatgcacgagcgcatggacgatgaaaacctggacgtcgacgagaattgcgtgctggttttgaagaattgcgggccccgcggctatccgggtatggccgaagccggcaatatgccgctgccgccgaaaatcctgcgcaaaggcatcaccgatatggtccgggtgtccgacgcccgcatgagcggcaccgcgtatggcacggtggttctgcatgtggcccccgaggccgccgcgggcggccctttggcgctggtgcaggacggcgacatcatcgaactggatgtggccgcgcgcaagctgcatttgcatgtgtccgatgaagagctcgcacgccgccgcgaggcatggcaagcgccgccggcgcccatggcgcgcggctgggtcaagctttatgtcgagcatgtgcagcaagccaatctgggcgccgaccttgattttctgcgaggtaaaagcggcgcgggcatacccaaagacaatcactga

SEQ ID NO: 11 - protein, 303 aa, Variovorax paradoxus B4
MDALELKNIVSDGLLSFPVTDFDQNGDFNAASYAKRLEWLAPYGASALFAAGGTGEFFSLTGDEYSDVIKTAVDACKGSVPIIAGAGGPTRQAILQAQEAERLGAHGILLMPHYLTEASQEGLVEHVKQVCNAVNFGVIFYNRSVSKLNVDSLQQLVESCPNLIGFKDSSGQIDMMTEVVQTLGDRLSYLGGLPTAEIFAAPYKALGSPVYSSAVFNFIPKTAMEFYNALRNDDFATTQRLIRDFFLPLIKIRNRKSGYAVSMVKAGAKIVGHDAGPVRPPLSDLTPQDYEDLAALIATLGPQ

SEQ ID NO: 12 - DNA, 1444 bp, Variovorax paradoxus B4
  source 1..1444: mol_type = genomic DNA
atgaccgccacctacaccgacacccgcctgctgatcgacaacgaatgggtcgacgccaccggcggcaagacgctggacgtcgtgaaccccgccaccggcaaagtcatcggcaaggtggcgcatgccagcatcgccgacctggaccgcgccctggccgccgcccagcgcggcttcgacaaatggcgcaacacccccgccaacgagcgcgccgccgtcatgcgccgcgcagccggcctcatccgcgaacgcgccggcgacatcgccaagctgctgacgcaagagcagggcaagccgctcgccgaagccaagggcgagaccctggccgccgccgacatcatcgaatggttcgccgacgaaggccgccgcgtctacggccgcatcgtgccctcgcggaacctggccgcgcagcagctcgtgctcaaggagccgctcggccccgtcgcagcgttcacgccgtggaacttcccgatcaaccagatcgtgcgcaagctcggcgcagcgctggccaccggctgctcgttcctggtgaaggcgcccgaagaaaccccggcgtcccccgccgcgctgctgcaggctttcgtcgacgcaggcattccgcccggcaccgtcggcctcgtgttcggcaaccccgctgaaatctcgaactacctcattgcccacccgatcatccgcaaggtcaccttcaccggctcgaccccggtcggcaagcagctggccgcgctggccggctcgcacatgaagcgcgtcacgatggagctgggcggccacgccccggtgatcgtggccgaagacgccgacgttgccctggccgtcaaggccgccggcgccgccaagttccgcaatgccggccaggtctgcatttcgccgacccgcttcctggtgcacaacagcctgcgcgaagagttcgcccgcacgctggtcaagtacaccgaaggcctgaagctcggcgacggcctcgccgaaggcaccaccatcggcccgctggccaacgcacgccgcctcaccgcgatggcctacgtgctggaagacgcgcgcaagaagggcgccacagtggcggccggcggcgaacgcgtcggcgactcgggcaactttttcgcgcccaccgtgctgaccgacgtgccgctggacgccgacgtgttcaacaacgagcccttcggccccatcgccgcgatccgtggcttcgacacgctcgaagaagcgatcgccgaagccaaccgcctgccattcggcctggccggctacgccttcaccaagtcgatcaagagcgcccacctgctgagccagaagctcgaactcggcatgctgtggatcaaccagcccgccaccccgtcgccggaaatgccgttcggcggcgtgaaggattcgggctacggttcggaaggcggccccgaggcgctcgaggcttacctgaacaccaaggccgtgtcgatcctcggcgtttaaa

SEQ ID NO: 13 - protein, 550 aa, Lactococcus lactis
MASMYTVGDYLLDRLHELGIEEIFGVPGDYNLQFLDQIISREDMKWIGNANELNASYMADGYARTKKAAAFLTTFGVGELSAINGLAGSYAENLPVVEIVGSPTSKVQNDGKFVHHTLADGDFKHFMKMHEPVTAARTLLTAENATYEIDRVLSQLLKERKPVYINLPVDVAAAKAEKPALSLEKESSTTNTTEQVILSKIEESLKNAQKPVVIAGHEVISFGLEKTVTQFVSETKLPITTLNFGKSAVDESLPSFLGIYNGKLSEISLKNFVESADFILMLGVKLTDSSTGAFTHHLDENKMISLNIDEGIIFNKVVEDFDFRAVVSSLSELKGIEYEGQYIDKQYEEFIPSSAPLSQDRLWQAVESLTQSNETIVAEQGTSFFGASTIFLKSNSRFIGQPLWGSIGYTFPAALGSQIADKESRHLLFIGDGSLQLTVQELGLSIREKLNPICFIINNDGYTVEREIHGPTQSYNDIPMWNYSKLPETFGATEDRVVSKIVRTENEFVSVMKEAQADVNRMYWIELVLEKEDAPKLLKKMGKLFAEQNK

SEQ ID NO: 14 - DNA, 1644 bp, Lactococcus lactis
  source 1..1644: mol_type = other DNA
atgtatacagtaggagattacctgttagaccgattacacgagttgggaattgaagaaatttttggagttcctggtgactataacttacaatttttagatcaaattatttcacgcgaagatatgaaatggattggaaatgctaatgaattaaatgcttcttatatggctgatggttatgctcgtactaaaaaagctgccgcatttctcaccacatttggagtcggcgaattgagtgcgatcaatggactggcaggaagttatgccgaaaatttaccagtagtagaaattgttggttcaccaacttcaaaagtacaaaatgacggaaaatttgtccatcatacactagcagatggtgattttaaacactttatgaagatgcatgaacctgttacagcagcgcggactttactgacagcagaaaatgccacatatgaaattgaccgagtactttctcaattactaaaagaaagaaaaccagtctatattaacttaccagtcgatgttgctgcagcaaaagcagagaagcctgcattatctttagaaaaagaaagctctacaacaaatacaactgaacaagtgattttgagtaagattgaagaaagtttgaaaaatgcccaaaaaccagtagtgattgcaggacacgaagtaattagttttggtttagaaaaaacggtaactcagtttgtttcagaaacaaaactaccgattacgacactaaattttggtaaaagtgctgttgatgaatctttgccctcatttttaggaatatataacgggaaactttcagaaatcagtcttaaaaattttgtggagtccgcagactttatcctaatgcttggagtgaagcttacggactcctcaacaggtgcattcacacatcatttagatgaaaataaaatgatttcactaaacatagatgaaggaataattttcaataaagtggtagaagattttgattttagagcagtggtttcttctttatcagaattaaaaggaatagaatatgaaggacaatatattgataagcaatatgaagaatttattccatcaagtgctcccttatcacaagaccgtctatggcaggcagttgaaagtttgactcaaagcaatgaaacaatcgttgctgaacaaggaacctcattttttggagcttcaacaattttcttaaaatcaaatagtcgttttattggacaacctttatggggttctattggatatacttttccagcggctttaggaagccaaattgcggataaagagagcagacaccttttatttattggtgatggttcacttcaacttaccgtacaagaattaggactatcaatcagagaaaaactcaatccaatttgttttatcataaataatgatggttatacagttgaaagagaaatccacggacctactcaaagttataacgacattccaatgtggaattactcgaaattaccagaaacatttggagcaacagaagatcgtgtagtatcaaaaattgttagaacagagaatgaatttgtgtctgtcatgaaagaagcccaagcagatgtcaatagaatgtattggatagaactagttttggaaaaagaagatgcgccaaaattactgaaaaaaatgggtaaattatttgctgagcaaaataaatag

SEQ ID NO: 15 - protein, 558 aa, Acetobacter pasteurianus
MTYTVGMYLAERLVQIGLKHHFAVAGDYNLVLLDQLLLNKDMKQIYCCNELNCGFSAEGYARSNGAAAAVVTFSVGAISAMNALGGAYAENLPVILISGAPNSNDQGTGHILHHTIGKTDYSYQLEMARQVTCAAESITDAHSAPAKIDHVIRTALRERKPAYLDIACNIASEPCVRPGPVSSLLSEPEIDHTSLKAAVDATVALLEKSASPVMLLGSKLRAANALAATETLADKLQCAVTIMAAAKGFFPEDHAGFRGLYWGEVSNPGVQELVETSDALLCIAPVFNDYSTVGWSAWPKGPNVILAEPDRVTVDGRAYDGFTLRAFLQALAEKAPARPASAQKSSVPTCSLTATSDEAGLTNDEIVRHINALLTSNTTLVAETGDSWFNAMRMTLPRGARVELEMQWGHIGWSVPSAFGNAMGSQDRQHVVMVGDGSFQLTAQEVAQMVRYELPVIIFLINNRGYVIEIAIHDGPYNYIKNWDYAGLMEVFNAGEGHGLGLKATTPKELTEAIARAKANTRGPTLIECQIDRTDCTDMLVQWGRKVASTNARKTTLA

SEQ ID NO: 16 - DNA, 1677 bp, Acetobacter pasteurianus
  source 1..1677: mol_type = other DNA
atgacctataccgttggtatgtatctggcagaacgtctggttcagattggtctgaaacatcattttgcagttgccggtgattataacctggttctgctggatcagctgctgctgaataaagatatgaagcagatttattgctgcaacgaactgaattgtggttttagtgccgaaggttatgcacgtagcaatggtgcagcagccgcagttgttacctttagcgttggtgcaattagcgcaatgaatgcattaggtggtgcctatgcagaaaatctgccggttattctgattagtggtgcaccgaatagcaatgatcaaggcaccggtcatattctgcatcataccattggtaaaaccgattatagctaccagctggaaatggcacgtcaggttacctgtgcagcagaaagcattaccgatgcacatagcgcaccggcaaaaattgatcatgttattcgtaccgcactgcgtgaacgtaaaccggcatatctggatattgcatgtaatattgcaagcgaaccgtgtgttcgtccgggtcctgttagcagcctgctgagcgaaccggaaatcgatcataccagcctgaaagcagcagttgatgcaaccgttgcactgctggaaaaaagcgcaagtccggtgatgctgctgggtagcaaactgcgtgcagcaaatgcactggcagcaaccgaaacactggcagataaactgcagtgtgcagttaccattatggcagcagcaaaaggtttttttccggaagatcatgcaggttttcgtggtctgtattggggtgaagttagcaatccgggtgttcaagaactggttgaaaccagtgatgccctgctgtgtattgcaccggtttttaatgattatagcaccgttggttggagcgcatggccgaaaggtccgaatgttattctggccgaaccggatcgtgttaccgttgatggtcgtgcatacgatggttttaccctgcgtgcctttctgcaggcactggccgaaaaagcaccggcacgtccggcaagcgcacagaaaagcagcgttccgacctgtagcctgaccgcaacctcagatgaagcaggtctgaccaatgatgaaattgtgcgtcatattaatgcgctgctgaccagcaataccacactggttgcagaaaccggtgatagctggtttaatgcaatgcgtatgaccctgcctcgtggtgcacgtgttgaactggaaatgcagtggggtcatattggttggtcagttccgagcgcatttggcaatgcaatgggtagccaggatcgtcagcatgttgttatggttggtgatggtagctttcagctgaccgcacaagaggttgcacagatggttcgttatgaactgcctgttattatcttcctgattaacaatcgcggttacgtgattgaaattgccattcatgatggtccgtacaactacatcaaaaactgggattatgccggtctgatggaagtgtttaatgccggtgaaggtcatggtctgggtctgaaagcaacaaccccgaaagaactgaccgaagcaattgcacgtgccaaagcaaatacccgtggtccgacactgattgaatgtcagattgatcgtaccgattgtaccgatatgctggttcagtggggacgtaaagttgcaagcaccaatgcacgtaaaacaaccctggcataa

SEQ ID NO: 17 - protein, 317 aa, Geobacillus stearothermophilus
MKNNGGARVVVIGAGFVGASYVFALMNQGIADEIVLIDANESKAIGDAMDFNHGKVFAPKPVDIWHGDYDDCRDADLVVICAGANQKPGETRLDLVDKNIAIFRSIVESVMASGFQGLFLVATNPVDILTYATWKFSGLPHERVIGSGTILDTARFRFLLGEYFSVAPQNVHAYIIGEHGDTELPVWSQAYIGVMPIRKLVESKGEEAQKDLERIFVNVRDAAYQIIEKKGATYYGIAMGLARVTRAILHNENAILTVSAYLDGLYGERDVYIGVPAVINRNGIREVIEIELNDDEKNRFHHSAATLKSVLARAFTR

SEQ ID NO: 18 - DNA, 954 bp, Geobacillus stearothermophilus
  source 1..954: mol_type = other DNA
atgaaaaacaacggtggagcccgagtagtggtcatcggcgccgggtttgtcggcgccagttatgtgtttgccttaatgaatcaagggattgccgatgagatcgtgctcatcgatgcgaatgaaagcaaggccataggcgatgcgatggacttcaaccatgggaaagtatttgcgccgaagccggttgacatttggcacggcgattacgatgattgccgcgatgccgatttggttgtcatttgcgccggcgccaaccaaaaaccgggcgagacgcggcttgatcttgtggacaaaaacattgccattttccgctcgatcgttgagtcggtcatggcatccggatttcaaggactgtttctcgtcgccaccaatccggtcgacattttaacgtacgcgacgtggaaattcagcggcctgccgcatgagcgggtgatcggttcggggacgattttagatacggcgcggttccgctttttgttgggcgagtatttctctgtcgctccgcaaaatgttcatgcctatattattggggaacacggcgacactgaactcccggtctggagccaggcttatatcggcgtcatgccgatccgcaagctggtcgagtccaaaggggaagaagcgcaaaaagatctcgagcgcatttttgtcaatgtgcgcgatgccgcctaccaaattattgagaaaaaaggagcgacgtactacgggattgcgatggggcttgcccgcgtgacgcgcgccattttgcataacgaaaacgctattttgaccgtatcagcctacctcgatggcctatatggggagcgcgacgtctacatcggagtgccggctgtcattaaccgcaatggcatccgcgaggtgatcgaaattgaattgaatgatgacgaaaaaaatcgattccatcatagcgcagctacattaaaaagcgtgctagcccgtgcttttacgcgatga

SEQ ID NO: 19 - protein, 339 aa, Geobacillus stearothermophilus
MKAAVVEQFKEPLKIKEVEKPTISYGEVLVRIKACGVCHTDLHAAHGDWPVKPKLPLIPGHEGVGIVEEVGPGVTHLKVGDRVGIPWLYSACGHCDYCLSGQETLCEHQKNAGYSVDGGYAEYCRAAADYVVKIPDNLSFEEAAPIFCAGVTTYKALKVTGAKPGEWVAIYGIGGLGHVAVQYAKAMGLNVVAVDIGDEKLELAKELGADLVVNPLKEDAAKFMKEKVGGVHAAVVTAVSKPAFQSAYNSIRRGGACVLVGLPPEEMPIPIFDTVLNGIKIIGSIVGTRKDLQEALQFAAEGKVKTIIEVQPLEKINEVFDRMLKGQINGRVVLTLEDK

SEQ ID NO: 20 - DNA, 1020 bp, Geobacillus stearothermophilus
  source 1..1020: mol_type = other DNA
atgaaagcagcagttgtggaacagtttaaagaaccgctgaaaatcaaagaggtggaaaaaccgaccattagctatggtgaagttctggttcgtattaaagcctgtggtgtttgtcataccgatctgcatgcagcacatggtgattggcctgttaaaccgaaactgccgctgattccgggtcatgaaggtgttggtattgttgaagaggttggtccgggtgttacccatctgaaagttggtgatcgtgttggtattccgtggctgtatagcgcatgtggtcattgtgattattgtctgagcggtcaagaaaccctgtgtgaacatcagaaaaatgcaggttatagcgtggatggtggttatgcagaatattgtcgtgcagcagcagattatgttgtgaaaattccggataacctgagctttgaagaagcagcaccgattttttgtgccggtgttaccacctataaagcactgaaagttaccggtgcaaaaccgggtgaatgggttgcaatttatggtattggtggtctgggccatgttgcagttcagtatgcaaaagcaatgggtctgaatgttgttgcagtggatatcggtgatgaaaaactggaactggcaaaagaactgggtgcagatctggttgttaatccgctgaaagaagatgcagccaaatttatgaaagaaaaagtgggtggtgttcatgcagcagttgttaccgcagttagcaaaccggcatttcagagcgcatataatagcattcgtcgtggtggtgcatgtgttctggttggtctgcctccggaagaaatgccgattccgatttttgataccgttctgaacggcattaaaatcattggtagcattgttggcacccgtaaagatctgcaagaagcactgcagtttgcagcagaaggtaaagttaaaaccatcattgaagttcagccgctggaaaaaatcaacgaagtttttgatcgcatgctgaaaggtcagattaatggtcgtgttgttctgaccctggaagataaataa

SEQ ID NO: 21 - protein, 378 aa, Bacillus subtilis
MIIGVPKEIKNNENRVALTPGGVSQLISNGHRVLVETGAGLGSGFENEAYESAGAEIIADPKQVWDAEMVMKVKEPLPEEYVYFRKGLVLFTYLHLAAEPELAQALKDKGVTAIAYETVSEGRTLPLLTPMSEVAGRMAAQIGAQFLEKPKGGKGILLAGVPGVSRGKVTIIGGGVVGTNAAKMAVGLGADVTIIDLNADRLRQLDDIFGHQIKTLISNPVNIADAVAEADLLICAVLIPGAKAPTLVTEEMVKQMKPGSVIVDVAIDQGGIVETVDHITTHDQPTYEKHGVVHYAVANMPGAVPRTSTIALTNVTVPYALQIANKGAVKALADNTALRAGLNTANGHVTYEAVARDLGYEYVPAEKALQDESSVAGA

SEQ ID NO: 22 - DNA, 1137 bp, Bacillus subtilis
  source 1..1137: mol_type = genomic DNA
atgatcataggggttcctaaagagataaaaaacaatgaaaaccgtgtcgcattaacacccgggggcgtttctcagctcatttcaaacggccaccgggtgctggttgaaacaggcgcgggccttggaagcggatttgaaaatgaagcctatgagtcagcaggagcggaaatcattgctgatccgaagcaggtctgggacgccgaaatggtcatgaaagtaaaagaaccgctgccggaagaatatgtttattttcgcaaaggacttgtgctgtttacgtaccttcatttagcagctgagcctgagcttgcacaggccttgaaggataaaggagtaactgccatcgcatatgaaacggtcagtgaaggccggacattgcctcttctgacgccaatgtcagaggttgcgggcagaatggcagcgcaaatcggcgctcaattcttagaaaagcctaaaggcggaaaaggcattctgcttgccggggtgcctggcgtttcccgcggaaaagtaacaattatcggaggaggcgttgtcgggacaaacgcggcgaaaatggctgtcggcctcggtgcagatgtgacgatcattgacttaaacgcagaccgcttgcgccagcttgatgacatcttcggccatcagattaaaacgttaatttctaatccggtcaatattgctgatgctgtggcggaagcggatctcctcatttgcgcggtattaattccgggtgctaaagctccgactcttgtcactgaggaaatggtaaaacaaatgaaacccggttcagttattgttgatgtagcgatcgaccaaggcggcatcgtcgaaactgtcgaccatatcacaacacatgatcagccaacatatgaaaaacacggggttgtgcattatgctgtagcgaacatgccaggcgcagtccctcgtacatcaacaatcgccctgactaacgttactgttccatacgcgctgcaaatcgcgaacaaaggggcagtaaaagcgctcgcagacaatacggcactgagagcgggtttaaacaccgcaaacggacacgtgacctatgaagctgtagcaagagatctaggctatgagtatgttcctgccgagaaagctttacaggatgaatcatctgtggcgggtgcttaa

SEQ ID NO: 23 - protein, 572 aa, Bacillus subtilis
MLTKATKEQKSLVKNRGAELVVDCLVEQGVTHVFGIPGAKIDAVFDALQDKGPEIIVARHEQNAAFMAQAVGRLTGKPGVVLVTSGPGASNLATGLLTANTEGDPVVALAGNVIRADRLKRTHQSLDNAALFQPITKYSVEVQDVKNIPEAVTNAFRIASAGQAGAAFVSFPQDVVNEVTNTKNVRAVAAPKLGPAADDAISAAIAKIQTAKLPVVLVGMKGGRPEAIKAVRKLLKKVQLPFVETYQAAGTLSRDLEDQYFGRIGLFRNQPGDLLLEQADVVLTIGYDPIEYDPKFWNINGDRTIIHLDEIIADIDHAYQPDLELIGDIPSTINHIEHDAVKVEFAEREQKILSDLKQYMHEGEQVPADWKSDRAHPLEIVKELRNAVDDHVTVTCDIGSHAIWMSRYFRSYEPLTLMISNGMQTLGVALPWAIGASLVKPGEKVVSVSGDGGFLFSAMELETAVRLKAPIVHIVWNDSTYDMVAFQQLKKYNRTSAVDFGNIDIVKYAESFGATGLRVESPDQLADVLRQGMNAEGPVIIDVPVDYSDNINLASDKLPKEFGELMKTKALL

SEQ ID NO: 24 - DNA, 1716 bp, Bacillus subtilis
  source 1..1716: mol_type = other DNA
atgctgaccaaagcaaccaaagaacagaaaagcctggtgaaaaatcgtggtgcagaactggttgttgattgtctggttgaacagggtgttacccatgtttttggtattccgggtgcaaaaattgatgcagtttttgatgccctgcaggataaaggtccggaaattattgttgcacgccatgaacagaatgcagcatttatggcacaggcagttggtcgtctgaccggtaaaccgggtgttgttctggttaccagcggtccgggtgcaagcaatctggcaaccggtctgctgaccgcaaataccgaaggtgatccggttgttgcactggcaggtaatgttattcgtgcagatcgtctgaaacgtacccatcagagcctggataatgcagcactgtttcagccgattaccaaatattcagttgaagtgcaggatgtgaaaaatattccggaagcagttaccaatgcctttcgtattgcaagcgcaggtcaggcaggcgcagcatttgttagctttccgcaggatgttgttaatgaagtgaccaataccaaaaatgttcgtgcagttgcagcaccgaaactgggtccggcagcagatgatgcaattagcgcagcaattgcaaaaattcagaccgcaaaactgccggttgttctggtgggtatgaaaggtggtcgtccggaagcaattaaagcagttcgtaaactgctgaaaaaagttcagctgccgtttgttgaaacctatcaggcagcaggcaccctgagccgtgatctggaagatcagtattttggtcgtattggtctgtttcgtaatcagcctggtgatctgctgctggaacaggcagatgttgttctgaccattggttatgatccgattgagtatgatccgaaattttggaacattaatggcgatcgcaccattattcacctggatgaaattattgccgatatcgatcatgcatatcagccggatctggaactgattggtgatattccgagcaccattaaccatattgaacatgatgccgtgaaagtggaatttgcagaacgtgaacagaaaattctgagcgatctgaaacagtatatgcatgaaggtgaacaggttccggcagattggaaaagcgatcgtgcacatccgctggaaattgttaaagaactgcgtaatgccgtggatgatcatgttaccgttacctgtgatattggtagccatgcaatttggatgagccgttattttcgtagctatgaaccgctgaccctgatgattagcaatggtatgcagaccctgggtgttgcactgccgtgggcaattggtgcaagcctggttaaaccgggtgaaaaagttgttagcgttagcggtgatggtggttttctgtttagcgcaatggaactggaaaccgcagttcgtctgaaagcaccgattgttcatattgtttggaacgatagcacctatgatatggttgcatttcagcagctgaaaaaatataatcgtaccagcgcagtggattttggcaatattgacattgtgaaatacgccgaaagctttggtgccaccggtctgcgtgttgaaagtccggatcagctggcagatgttctgcgtcagggtatgaatgcagaaggtccggttattattgatgttccggttgattatagcgataacattaatctggccagcgataaactgccgaaagaatttggtgaactgatgaaaaccaaagccctgtta

SEQ ID NO: 25 - protein, 367 aa, Geobacillus stearothermophilus
MELFKYMETYDYEQVLFCQDKESGLKAIIAIHDTTLGPALGGTRMWMYNSEEEALEDALRLARGMTYKNAAAGLNLGGGKTVIIGDPRKDKNEAMFRAFGRFIQGLNGRYITAEDVGTTVADMDIIYQETDYVTGISPEFGSSGNPSPATAYGVYRGMKAAAKEAFGSDSLEGKVVAVQGVGNVAYHLCRHLHEEGAKLIVTDINKEVVARAVEEFGAKAVDPNDIYGVECDIFAPCALGGIINDQTIPQLKAKVIAGSADNQLKEPRHGDIIHEMGIVYAPDYVINAGGVINVADELYGYNRERAMKKIEQIYDNIEKVFAIAKRDNIPTYVAADRMAEERIETMRKARSPFLQNGHHILSRRRAR

SEQ ID NO: 26 - DNA, 1101 bp, Geobacillus stearothermophilus
  source 1..1101: mol_type = other DNA
atggaactgttcaaatacatggaaacctatgactatgaacaggtgctgttttgccaggataaagaaagcggtctgaaagccattattgccattcatgataccaccctgggtccggcactgggtggcacccgtatgtggatgtataatagcgaagaagaagcactggaagacgccctgcgtctggcacgtggtatgacctataaaaacgcagcagcaggtctgaatctgggtggtggtaaaaccgttattattggtgatccgcgtaaagataaaaacgaagccatgtttcgtgcctttggtcgttttattcagggtctgaatggtcgttatattaccgcagaagatgttggcaccaccgttgcagatatggatattatctatcaagaaaccgattacgtgaccggtattagtccggaatttggtagcagcggtaatccgagtccggcaaccgcctatggtgtttatcgcggtatgaaagcagcagcaaaagaagcctttggtagcgatagcctggaaggtaaagttgttgcagttcagggtgttggtaatgttgcatatcatctgtgtcgtcatctgcatgaagaaggtgcaaaactgattgtgaccgatatcaataaagaagttgtggcacgcgcagttgaagaatttggtgcaaaagcagttgatccgaacgatatttatggtgtggaatgcgatatttttgcaccgtgtgcactgggaggtattatcaatgatcagaccattccgcagctgaaagcaaaagttattgcaggtagcgcagataaccaactgaaagaaccgcgtcatggtgatattattcatgaaatgggtattgtgtatgcaccggactatgttattaatgccggtggtgtgattaatgttgccgatgaactgtatggttataatcgtgaacgtgccatgaaaaaaatcgagcagatctatgacaacatcgagaaagtttttgccattgccaaacgcgataatattccgacctatgttgcagcagatcgtatggcagaagaacgtattgaaaccatgcgtaaagcacgtagcccgtttctgcaaaatggtcatcatattctgagccgtcgtcgtgcacgc

SEQ ID NO: 27 - protein, 259 aa, Cohaesibacter celericrescens
MPKFAANLSMMFTELDFLDRFEAAAKAGFKGVEYLFPYDFDKDELAGLLKANGLKQVLHNLPAGNWAAGERGIACLPDRVGEFKDGVGQAIDYAKALGCPQLNCLAGKIPDGVSPEEAHSTLVANLTFAAEELSKAGIKLLVEPINHFDIPGFAVTTSTQGLAIISAVGSDNLFLQYDIYHMQRMEGELANTMQANLALIRHIQLADNPGRHEPGTGEINYSFLFRFLDQIGYDGWIGCEYAPANGTEAGLGWLAPYQS

SEQ ID NO: 28 - DNA, 780 bp, Cohaesibacter celericrescens
  source 1..780: mol_type = other DNA
atgccaaaattcgcagccaatttatcaatgatgttcacggaattagatttcttagaccgattcgaggccgcggccaaagccggcttcaagggtgtggagtaccttttcccgtacgatttcgacaaggacgagcttgcgggcctgcttaaggctaacgggctgaaacaagtcctgcacaaccttccggctggaaattgggccgctggagagcgtggcatagcctgcctgcctgaccgtgtgggagaatttaaggatggtgtaggacaagccatagactacgccaaagcattaggttgcccccaactgaattgcttggcagggaagatccctgatggagtttcgccggaagaggcccacagcacccttgttgcaaacctgacttttgcagcagaggagctgtccaaggcggggataaaattactcgtagaaccgatcaatcattttgatatacctgggttcgcagttaccacttcgacacaaggtcttgcaatcatttccgcggtaggtagtgataacctctttctccaatacgatatctaccacatgcaacgcatggaaggcgagttggccaatactatgcaagccaacctggccctgatccgacacattcagttggctgacaatcctggacgccacgaaccgggcacgggtgagataaactattctttcttatttcgatttctggaccaaattggatatgacggctggatcggctgcgagtacgcgcccgcaaatggtactgaggcaggcttgggctggcttgcaccctatcaaagttga

SEQ ID NO: 29 - protein, 259 aa, Polynucleobacter wuianus
MPKFAANLTMLFNEVPFLDRFEKASSAGFKAVEFLFPYPFAANEIKQKLDQNQLSLVLHNLPAGDWDAGERGIACLPDRKEEFRAGVAKAIEYAKVLGVHQLNCLAGKVPTGADQKLAHATFVENLRYAAAELKKNHLRLLIEPINTFDIPGFFLNITQQAIDILSEVGADNVFVQYDIYHAQRMEGELANTIEKHFEKIAHIQLADNPGRNEPGTGEINYAYLFNHLDRIGYKGWIGCEYKPATTTEAGLGWIKQFNS

SEQ ID NO: 30 - DNA, 780 bp, Polynucleobacter wuianus
  source 1..780: mol_type = other DNA
atgccaaagtttgccgcgaacctgacaatgttgttcaatgaggtaccatttctcgaccgctttgagaaggctagctctgctggtttcaaggctgtagagttccttttcccgtatccgttcgctgccaatgagatcaaacaaaagttggaccagaaccaattatccttggttcttcacaatctcccagcgggcgactgggacgcgggtgaacgaggaatcgcttgtctcccagatcgcaaagaggagttccgggcgggtgtcgctaaagccatagagtacgctaaggtactgggtgtgcatcaattaaactgcttagcgggaaaagtaccaactggcgcagaccaaaagttggctcatgctacgttcgtcgaaaacttacgttacgctgccgccgagttaaagaagaaccacttgagattactcattgagcctattaatacattcgacatcccggggttcttccttaatataacccaacaagccattgacatactgagcgaagtgggtgctgataacgtcttcgtccaatacgatatctaccacgcacaaagaatggaaggggaattagccaacactattgaaaagcacttcgaaaagatagcccacatacaactggctgacaaccctggtcgtaatgaacctgggacgggtgaaattaactacgcatatctcttcaatcacctcgatagaataggttataagggatggataggatgcgaatataagccggccactacgaccgaggctggtttaggttggataaaacagttcaactcatga

SEQ ID NO: 31 - protein, 264 aa, Sulfobacillus acidophilus DSM 10332
MLKFAANLTMLYGDSPFLERFDRARQSGFDFVEFLFPYGAGLSAVEKARQDAQLTIVLFNLPAGDWDQGERGIAIFPDRRAEFREGVAEAIRYAKALGVSQVNCLAGRRPEDLPVDEAWAVLRENVRYAADALEREGLTLLMEPINPFDVPGFFINSPREVMRLREETGVPNLRLQYDIYHQQRTAGEILATFHAFRASVGHIQIADNPGRHQPGTGELHYGRIFSALDSAGYSGYIGLEYIPDGTTEESLEWWRQYQAGQFLG

SEQ ID NO: 32 - DNA, 795 bp, Sulfobacillus acidophilus DSM 10332
  source 1..795: mol_type = other DNA
atgctcaaattcgcggcgaacttaactatgctctatggtgacagcccgttcttagagcgcttcgaccgagcacgccaaagtggtttcgatttcgtcgagtttctcttcccgtatggagcgggtctgtccgccgtagagaaggcccgtcaggatgcccaacttacgattgtgctcttcaacctgcctgctggggactgggatcaaggagaaagaggaatagcaatattccctgacagaagagccgaatttcgcgagggtgttgcggaagcgatccgttacgcaaaagcccttggagtctcacaagtcaactgtttggctggccgacgccccgaggacctgccggtcgatgaggcctgggctgttttacgcgagaacgttcggtacgctgcagatgcacttgagcgcgaaggtcttacactcctcatggagccgatcaaccctttcgacgtcccgggtttcttcataaacagtcctcgcgaggttatgcgacttagagaagagacaggtgtacctaaccttcgcttacaatacgacatctaccaccagcaaagaactgccggggaaatcttagccaccttccatgcctttcgcgcttcggtggggcatatccaaattgcggacaaccctggacgccaccagcccggaacgggcgagctgcattacggccgcatattcagcgcacttgactcagccggttactccgggtacattggtttagagtacattcctgatggcaccacggaagagagtctggaatggtggcgacagtaccaagcaggacaatttctcggctga

SEQ ID NO: 33 - protein, 264 aa, Sulfobacillus thermosulfidooxidans DSM 9293
MLKFAANLTMLYTDVPFLERFGRARVSGFDAVEFLFPYSDGLDAVTTVAREAAVTIALFNLPAGDWEHGERGIAILPDRRAEFRAGVAEAIRYATALGVQRLNCLAGRRPDDLPEVEAWAVLRDNVRYAADELAKAHLTLMLEPINPYDIPGFFLNRTSEVIDLIREVGRSNIQIQYDIYHLQRTQGEIIGTFRTLREHIGHIQIADNPGRHQPGTGELNYKRIFSALDEAGYTGYIGLEYIPQGRTEDSLEWWRLYQNGQFAG

SEQ ID NO: 34 - DNA, 795 bp, Sulfobacillus thermosulfidooxidans DSM 9293
  source 1..795: mol_type = other DNA
atgttaaaattcgccgctaatctgaccatgctttacacggacgtaccgttcttggagcggttcgggcgtgccagagtgtctggcttcgatgcagtggagtttctgtttccttactcagacgggctggacgcagttaccactgtagcgcgagaggcggccgttaccattgccttgtttaacctgcctgctggcgactgggagcatggcgaacgtggcatcgcaatattgccagaccgacgtgctgagttcagagccggagttgcggaagccatccgctacgcgacggctctgggcgtgcaacgtttaaattgtctggccgggcggcgtccagatgaccttccagaggttgaagcatgggctgttttgcgcgataacgtccgttatgcggcagacgagctcgctaaagcccacttaacgctgatgctggaaccgatcaatccttacgatattccaggattctttctgaaccggacgagtgaggtaattgatctcattcgcgaggttggccgatccaacattcagattcagtacgatatatatcacttgcagcgcacgcaaggggaaattataggcaccttccggacgcttcgtgagcacataggtcatatccagatcgctgacaacccggggcggcatcaaccaggtaccggtgagcttaactacaagagaattttcagcgcgcttgacgaggcaggttatacaggctatataggacttgaatacattccccagggaagaacagaagattcccttgaatggtggcggttataccagaacgggcaatttgccgggtga

SEQ ID NO: 35 - protein, 260 aa, Pseudomonas putida DSM 6125
MPRFAANLSMLFTEQDFLARFKAAADAGFSGVEYLFPYDFSAADIKQQLEANGLTQVLFNLPAGDWAKGERGITCHPDRIEEFRAGVDKAIEYAKVLGNTQVNALAGIRPQGPDCATVRKTFVENLRYAADKLKGAGIRLVMEMINTRDIPGFYLNTTQQALEIQAEVGSDNLFLQYDIYHMQIMEGDLARTMEANLKLINHIQLADNPGRNEPGTGEINYRFLFEHLDRIGYQGWVGAEYKPLTTTEAGLGWLKTHNAI

SEQ ID NO: 36 - DNA, 783 bp, Pseudomonas putida DSM 6125
  source 1..783: mol_type = genomic DNA
atgcctcgcttcgctgccaacctgtccatgctgttcaccgaacaggacttcctggcccgcttcaaggctgccgccgatgctggtttcagcggcgtcgaatacctgttcccgtacgacttcagcgctgccgacatcaagcagcagctggaggccaacggcctgacccaggtgctgttcaacctgccggccggcgactgggccaaaggtgagcgcggtatcacctgccaccccgaccgcatcgaagagttccgtgccggtgtcgacaaggccatcgagtacgccaaggtgctgggcaatactcaggtcaacgccctggccggcatccgcccacaaggcccggactgcgccaccgtgcgtaagaccttcgtcgagaacctgcgctacgccgctgacaagctcaagggcgccgggatccgcctggtcatggaaatgatcaacacccgcgacatccccggcttctacctgaacaccacccagcaggccctggaaatccaggccgaagtgggcagcgacaacctgttcctgcaatacgacatctaccacatgcagatcatggaaggtgacctggctcgcaccatggaagccaacctgaagctgatcaaccacatccagctggccgacaacccaggccgcaatgaaccaggcaccggcgagatcaactaccgcttcctgttcgaacacctggaccgcattggctaccagggctgggtgggcgcggagtacaagccgctgaccaccaccgaagcgggcctgggctggctgaaaacccacaacgcaatctga

SEQ ID NO: 37 - protein, 258 aa, Vibrio natriegens NBRC 15636
MAKFAANLTMLFTEVPFLERFEKAHQAGFKAVEYLFPYAYEVQDLADKMQQFGFEQALFNMPPGDWDAGEKGFAAIPGREDEFKASVDTALMYADKLNCKKVHAMSGIVDKQFTREQHVETFIANIRYAADKFAEHGIELMIEPLNSRDVPNYFIAHQREAVELIKQVNRPNVKLQLDLYHAQIMDGDLSTLIREVAPYTGHIQIASVPERHEPSEGELNYPHLFGVLDDSGYQGWIGCEYNPRNTTEEGLDWVKPYL

SEQ ID NO: 38 - DNA, 777 bp, Vibrio natriegens NBRC 15636
  source 1..777: mol_type = genomic DNA
atggctaagtttgcagcaaatctcaccatgctatttacagaagtaccatttctggaacgttttgaaaaagcgcatcaagcgggatttaaagcggtggaatacctttttccttacgcttatgaagtgcaggatctggcagacaaaatgcagcaatttggattcgaacaagccctgttcaacatgcctcctggtgactgggatgctggcgaaaaaggctttgcagcaatccctggccgcgaagatgagtttaaagccagtgtagacaccgcgttaatgtatgccgacaagctgaattgcaaaaaggtacacgcgatgtcaggcatcgttgataagcaatttactcgcgagcaacatgtagaaacgtttatcgccaacattcgttatgcagcagacaagtttgctgagcatggcattgagctcatgatcgagccgctaaatagccgtgacgttcccaactacttcatcgctcatcagcgtgaagctgttgagttaattaagcaagtaaaccgaccaaatgtgaagctgcaactggatctttaccacgcacaaattatggacggtgatttaagcacgcttatccgtgaggttgcgccgtatacgggtcatattcaaatcgcgtcagtgccagaaagacacgagccttctgaaggagaactgaactatccgcatctgttcggtgttttagacgactcaggttatcagggctggatcggttgtgaatacaacccaagaaacactacagaggaaggactcgattgggttaagccgtatctgtaa

SEQ ID NO: 39 - protein, 260 aa, Cupriavidus necator DSM 13513
MTKLAANLTMLFNEVGFLDRFEAAARAGFRGVEFLFPYAFHADQIADRLNRFQLDLVLHNLPAGKWEAGERGIACHPDRVGEFQDGVGEAIKYAKVLGVRQLNCLVGIQPQNVKREQAQETLVENLRFAASALAAEHIDLLVEPINTFDIPGFFLSRTQQAVDLINQVNAPNLYVQYDIYHMQRMEGEIANTIKANLPKIKHVQLADNPGRNEPGTGELNYRFLFKFLDEIGYNGWIGCEYKPKTTTEAGLGWRAEHGVQ

SEQ ID NO: 40 - DNA, 783 bp, Cupriavidus necator DSM 13513
  source 1..783: mol_type = genomic DNA
atgactaaacttgcggccaacctcaccatgctgttcaatgaagtcggttttctcgaccgcttcgaagccgccgcgcgcgcgggcttccgcggcgtggaattcctcttcccctatgccttccatgcggatcagatcgctgaccgcctgaaccgcttccagctggacctggtgctgcacaacctgcccgccggcaagtgggaagcgggcgagcgcggcattgcctgccacccggaccgcgtcggcgagttccaggacggcgtgggcgaggccatcaagtacgccaaggtgctgggcgtgcgccagctgaactgcctggtcggcatccagccgcagaacgtcaagcgcgagcaggcccaggaaacgctggtggaaaacctgcgcttcgccgccagcgcgctcgctgctgagcatatcgacctgctggtcgagccgatcaacaccttcgacatccccggcttcttcctgtcgcgcacgcagcaggcggtggacctgatcaaccaggtcaatgcgcccaacctgtacgtgcagtacgacatctaccacatgcagcggatggaaggcgagatcgccaacaccatcaaggccaacctgccgaagatcaagcacgtgcagctggccgacaacccgggccgcaatgaaccggggaccggcgagctgaactaccgcttcctgttcaagttcctggacgagatcggctacaacggctggatcggctgcgagtacaagccgaagaccaccaccgaagccggcctgggctggcgcgccgagcacggcgtgcagtaa

SEQ ID NO: 41 - protein, 576 aa, Pseudomonas fluorescens
MAMITGGELVVRTLIKAGVEHLFGLHGIHIDTIFQACLDHDVPIIDTRHEAAAGHAAEGYARAGAKLGVALVTAGGGFTNAVTPIANARTDRTPVLFLTGSGALRDDETNTLQAGIDQVAMAAPITKWAHRVMATEHIPRLVMQAIRAALSAPRGPVLLDLPWDILMNQIDEDSVIIPDLVLSAHGAHPDPADLDQALALLRKAERPVIVLGSEASRTARKTALSAFVAATGVPVFADYEGLSMLSGLPDAMRGGLVQNLYSFAKADAAPDLVLMLGARFGLNTGHGSGQLIPHSAQVIQVDPDACELGRLQGIALGIVADVGGTIEALAQATAQDAAWPDRGDWCAKVTDLAQERYASIAAKSSSEHALHPFHASQVIAKHVDAGVTVVADGGLTYLWLSEVMSRVKPGGFLCHGYLNSMGVGFGTALGAQVADLEAGRRTILVTGDGSVGYSIGEFDTLVRKQLPLIVIIMNNQSWGWTLHFQQLAVGPNRVTGTRLENGSYHGVAAAFGADGYHVDSVESFSAALAQALAHNRPACINVAVALDPIPPEELILIGMDPFAGSTENLYFQSGAL

SEQ ID NO: 42 - DNA, 1725 bp, Pseudomonas fluorescens
  source 1..1725: mol_type = other DNA
atggctatgattactggtggtgaactggttgttcgtaccctgattaaagctggcgtagaacatctgtttggcctgcatggcattcatattgacaccatttttcaggcttgcctggaccacgacgtcccaatcattgatactcgccacgaagcggcggcaggccacgctgcggaaggttatgcccgcgcgggcgctaaactgggtgttgccctggtgaccgctggcggtggctttaccaatgccgttacgccgatcgcgaacgctaggaccgatcgcactccggttctgttcctgaccggttctggtgctcttcgtgatgacgaaaccaacaccctgcaggccggtattgatcaggtggcgatggcggccccgatcacgaaatgggctcatcgtgttatggcaactgaacacatcccgcgtctggttatgcaggccattcgtgccgctctgagcgccccacgtggcccggtgctgctggatctgccttgggacatcctgatgaaccaaatcgatgaagattccgttatcatcccagacctggtgctgtctgctcacggtgcccatccagacccggctgacctggaccaggctctggcactgctgcgtaaagccgaacgcccagttatcgtactgggctccgaggcgtcccgcaccgcacgcaagaccgcactgagcgcattcgtagcggcgaccggtgtaccggttttcgctgactatgaaggcctgtccatgctgagcggcctgccggacgctatgcgtggcggcctggtgcagaacctgtactcctttgcaaaagctgatgcagctccggacctggtactgatgctgggtgctcgtttcggtctgaacaccggtcatggttccggtcaactgatcccgcattctgctcaggtgatccaggtggacccagacgcgtgtgaactgggtcgcctgcaaggcatcgcgctgggtatcgtggctgatgtaggtggcaccattgaagcgctggctcaagcaactgcacaagatgcagcgtggccggaccgcggcgactggtgcgccaaggtaactgacctggcccaggagcgttacgcttccatcgcggctaaatccagctctgaacatgcgctgcacccgttccacgcttctcaggttatcgcgaaacacgtggacgcaggcgtgaccgtcgttgcggatggtggcctgacttatctgtggctgtccgaagttatgtctcgtgtcaaaccaggcggcttcctgtgccacggctatctgaacagcatgggtgtaggcttcggtactgccctgggtgcgcaggttgcggatctggaggcaggtcgtcgtaccatcctggtgaccggcgacggctctgttggttattccattggcgaattcgacaccctggtacgcaaacagctgccgctgattgtaattatcatgaacaaccagtcttggggctggaccctgcactttcagcagctggccgttggtcctaaccgtgtcaccggcacccgcctggaaaatggttcctatcacggcgttgctgcggcattcggtgctgatggttaccacgtcgactctgtcgagagcttcagcgccgctctggctcaggcactggcacacaaccgcccggcctgcatcaacgttgctgtggccctggacccgatcccgccggaggaactgatcctgattggcatggacccgtttgcgggctccacggagaatctgtatttccaatccggcgcg

SEQ ID NO: 43 - protein, 258 aa, Escherichia coli
MPRFAANLSMMFTEVPFIERFAAARKAGFDAVEFLFPYNYSTLQIQKQLEQNHLTLALFNTAPGDINAGEWGLSALPGREHEAHADIDLALEYALALNCEQVHVMAGVVPAGEDAERYRAVFIDNIRYAADRFAPHGKRILVEALSPGVKPHYLFSSQYQALAIVEEVARDNVFIQLDTFHAQKVDGNLTHLIRDYAGKYAHVQIAGLPDRHEPDDGEINYPWLFRLFDEVGYQGWIGCEYKPRGLTEEGLGWFDAWR

SEQ ID NO: 44 - DNA, 777 bp, Escherichia coli
  source 1..777: mol_type = genomic DNA
atgcctcgttttgcagctaatttatccatgatgttcaccgaagtgccttttattgaacgcttcgccgcagcgcgaaaagccgggttcgatgctgtggaatttctgtttccctataactactccaccctgcaaatccaaaagcaactggagcaaaaccatctgacactggcgctgttcaataccgctcccggagatattaatgcgggggaatggggattatccgcccttcccggacgtgagcacgaagcacacgcagacatcgacctggcactggaatatgcattggcgctcaattgtgaacaagtccatgtgatggcaggcgtcgtgcccgctggcgaagatgctgaacggtaccgggcagtatttatcgataatatccgctacgctgccgaccgctttgcgccacacggcaagcgaatattagttgaagcactcagccccggcgttaagcctcattatctcttctccagccagtatcaggcactggctattgttgaagaggttgcgcgagataacgtgtttattcaactagatacttttcatgcgcaaaaagtagatggcaacctgacgcatttaatccgcgactacgccgggaaatatgcgcacgtacaaattgccggactacctgatcgacatgaaccggacgatggagaaatcaactatccgtggctgttccgcctgttcgatgaggtgggatatcagggctggatcggttgtgaatataaacctcgtggcctcaccgaagaagggcttggctggtttgacgcctggcgctaa

SEQ ID NO: 45 - protein, 259 aa, Variovorax paradoxus
MPKFAANLTMLFTELPFMQRFEAAAKAGFKGVEYLFPYPFEKKELAAALRTNGLQQVLHNLPAGDWDKGERGIACLADRTGEFAEGIGMAIDYATALGCPQVNCLIGKVPEGADINVVNRTVIDNLRLAARELEAAGIRMLIEPINTFDIPGFYLNRTDKALALIEAVGSPNLKVQYDIYHAQRMEGELGNTLTKHLAQIGHIQLADNPGRGEPGTGEINYPWLFKHIDSLGYDGWIGCEYKPRSDTVNGLGWREALTQ

SEQ ID NO: 46 - DNA, 780 bp, Variovorax paradoxus
  source 1..780: mol_type = genomic DNA
atgcccaagttcgcagccaacctcacgatgctcttcaccgagctgccgttcatgcaacgcttcgaagccgccgccaaggcgggcttcaagggagtggaatacctcttcccgtaccccttcgagaagaaggaactcgccgcggcgctccgcaccaacggcctgcagcaggtgctgcacaacctgccggccggcgactgggacaagggcgagcgcggcatcgcgtgcctggccgaccgcaccggcgaattcgccgaaggcatcggcatggcgatcgactacgccaccgcgctcggctgcccgcaagtcaactgcctcatcggcaaggtgcccgagggcgccgacatcaatgtggtcaatcgcacggtgatcgacaacctgcgcctggccgcgcgggagctcgaggcggccggcatccgcatgctgatcgagccgatcaacaccttcgacattccgggcttctacctgaaccgcaccgacaaggcgctggcgctgatcgaggcggtgggctcgcccaacctgaaggtgcagtacgacatctatcacgcacagcgcatggaaggcgagctcggcaacacgctgaccaagcacctcgcgcagatcggccacatccagctggccgacaaccccggccgcggcgagccgggcacgggcgagatcaactatccgtggctcttcaagcacatcgattcgctgggctacgacggctggatcggctgcgaatacaagccgcgcagcgacacggtcaatggcctcggctggcgtgaagcgctcacgcaataa

SEQ ID NO: 47 - protein, 267 aa, Herbaspirillum seropedicae
MLRFAANLSMMYVEHDFLDRFAAAAKDGFSGVEFLFPYDYAPEEIKSRLEANGLTQALFNAPPGDWAAGERGIASLPGRQDEFKRSIETALKYAAVIGNQTLHVMAGLIKPGQDRAQHRAVYLDNLSYAAHQAESAGLTVVIEPINTRNIPGFFLNRQDDAQAICAEVGAPNLKVQFDCYHCQIVEGDVAVKLKRDMPGIGHIQIAGVPERHEPDVGELNYPYLLKLIDTLGYQGWIGCEYNPAGATSAGLGWLRALAEQGLTTLKK

SEQ ID NO: 48 - DNA, 804 bp, Herbaspirillum seropedicae
  source 1..804: mol_type = genomic DNA
atgctgcgttttgccgctaacctgagcatgatgtatgtggaacacgatttcctggaccgcttcgccgccgccgccaaggatggcttctccggcgtcgagttcctgttcccctatgactacgcgcctgaagagatcaagtcgcgcctggaggccaacggcctgacccaggcgctgttcaacgcgcccccgggcgactgggccgccggtgagcgcggtatcgcatcgctgccgggtcgccaggacgaattcaagcgcagcatcgagaccgcgctgaagtacgccgcagtgatcggcaaccagaccctgcacgtgatggccggcctgatcaagccgggccaggatcgcgcccagcatcgcgcggtctatctggacaacctgtcctatgccgcccaccaggccgagtccgctggcctgaccgtggtgatcgagccgatcaacacgcgcaacattcccggcttcttcctcaatcgccaggatgatgcgcaagccatctgcgccgaagtgggtgcgcccaacctgaaggtgcaattcgattgctaccactgccagatcgtcgaaggcgacgtggccgtgaagctcaagcgcgacatgcccggcatcggtcacatccagatcgccggtgtgcccgagcgccatgagccggacgtgggtgagctgaactatccgtatctgttgaagctgatcgataccctgggttaccagggatggattggttgcgagtacaacccggccggcgccacctcggctgggctggggtggttgagggcgctggcggagcagggtttgacgacgctgaagaagtga

SEQ ID NO: 49 - protein, 253 aa, Geobacillus stearothermophilus
MRKPIIAGNWKMHKTLAEAVQFVEDVKGHVPPADEVDSVVCAPFLFLDRLVQAADGTDLKIGAQTMHFADQGAYTGEVSPVMLKDLGVTYVILGHSERRQMFAETDETVNKKVLAAFTRGLIPIICCGESLEEREAGQTNAVVASQVEKALAGLTPEQVKQAVIAYEPIWAIGTGKSSTPEDANSVCGHIRSVVSRLFGPEAAEAIRIQYGGSVKPDNIRDFLAQQQIDGALVGGASLEPASFLQLVEAGRHE

SEQ ID NO: 50 - DNA, 762 bp, Geobacillus stearothermophilus
  source 1..762: mol_type = genomic DNA
atgagaaaaccgatcattgcaggcaactggaaaatgcataaaacattagcggaagcggttcaatttgtcgaggacgtaaaagggcacgtgccgccggccgacgaagtcgattccgtcgtttgcgcgccgtttctctttttggatcggttggtgcaagcggcagacggcacggatttaaaaatcggggcgcaaacgatgcactttgccgatcaaggggcgtacacaggcgaagtgagcccggtcatgctgaaagacctcggcgtcacgtacgtcatcctcggccattcggagcgccggcaaatgttcgccgaaacagatgagaccgtgaacaaaaaagtgttggccgccttcacccgcgggcttataccgattatttgctgcggtgaatcgcttgaggagcgggaagcggggcagacgaacgcggttgtcgcctcgcaagtggaaaaagcgctcgccggcttgacgccggaacaagtgaagcaagcggtcatcgcttacgagccgatttgggcgatcgggacgggcaaatcatcaacaccggaagacgccaacagcgtctgcggccatatccgttcggttgtttcgcgcctgtttggcccggaggcggcggaagcgatccgcattcaatacggcggcagcgtcaaaccagacaacatccgcgacttcttggcgcaacaacagatcgacggcgccttagtcggcggggcgagcctcgagccggcttcattcttgcaattggtggaggcggggcgtcatgagtaa

SEQ ID NO: 51 - protein, 341 aa, Geobacillus stearothermophilus
MAKFYYNGDANEQYLQGKTVAIIGYGSQGHAHAQNLRDSGVRVIVGLRKGKSWEQAEQDGFEVYSVREAAKQADIVMVLLPDEKQPAVYKEEIEPGLEPGNALVFAHGFNIHFSQIVPPEHVDVFLVAPKGPGHLVRRTYAEGAGVPALIAVYQDVTGHAKETALAYAKAIGAARAGVLETTFKEETETDLFGEQAVLCGGLTALIKAGFETLVEAGYQPEVAYFECLHEMKLIVDLLYEGGLSWMRYSISDTAQWGDFITGPRIINDAVKAEMKKVLDDIQTGKFAKSWILENQANRPEFNAINRRENEHLIEVVGRELRSMMPFVKAKQKKAVVPGAKH

SEQ ID NO: 52 - DNA, 1026 bp, Geobacillus stearothermophilus
  source 1..1026: mol_type = genomic DNA
atggcaaaattctactataacggggatgcaaacgaacaatatttgcaagggaaaacggtcgcgatcatcggctacggctcacaaggccacgcccatgcacaaaacttgcgcgacagcggcgtccgcgtcattgtcgggttgcgcaaagggaaatcgtgggagcaggcggaacaggacggctttgaagtatactcggtgcgcgaagcggcaaaacaagcggatattgtgatggtgttgctgccggatgagaaacagccggctgtctacaaggaagagattgaaccggggcttgaaccgggcaacgcgcttgtgtttgcgcacgggtttaacattcatttcagccaaatcgtcccgccggagcatgtcgatgtcttcttggtggcgccgaaaggaccaggccatctcgtgcgtcgcacatatgcggaaggagccggggtgccggcgctcatcgccgtttatcaagatgtaaccggacacgcgaaagaaacggcgctcgcctatgcgaaagcgattggtgctgctcgagctggggtgttggagacaacgttcaaagaagagacggaaaccgacttgttcggtgaacaagcggtgctgtgcggcgggctgacggcgctcatcaaggccgggtttgaaacgctcgttgaagccgggtatcagccggaagtcgcctatttcgagtgtttgcatgaaatgaagctcatcgttgatcttctttatgaaggtggcttgtcgtggatgcgctactcgatttccgatacggcgcaatggggcgactttatcaccggtccgcgcatcattaacgacgccgtgaaagcggaaatgaaaaaggtgctcgatgacatccaaaccggcaaattcgcgaaaagctggattttggaaaaccaagcaaaccgtccggagttcaacgccatcaaccggcgcgagaacgagcatttaatcgaagtcgtcggacgcgaactgcggagcatgatgccgtttgtgaaagcaaaacaaaaaaaagcggtggtgccaggtgcgaaacattaa

SEQ ID NO: 53 - protein, 413 aa, Escherichia coli
MKWFNTLSHNRWLEQETDRIFDFGKNSVVPTGFGWLGNKGQIKEEMGTHLWITARMLHVYSVAAAMGRPGAYSLVDHGIKAMNGALRDKKYGGWYACVNDEGVVDASKQGYQHFFALLGAASAVTTGHPEARKLLDYTIEIIEKYFWSEEEQMCLESWDEAFSKTEEYRGGNANMHAVEAFLIVYDVTHDKKWLDRAIRVASVIIHDVARNNHYRVNEHFDTQWNPLPDYNKDNPAHRFRAFGGTPGHWIEWGRLMLHIHAALEARCEQPPAWLLEDAKGLFNATVRDAWAPDGADGIVYTVDWEGKPVVRERVRWPIVEAMGTAYALYTVTGDRQYETWYQTWWEYCIKYLMDYENGSWWQELDADNKVTTKVWDGKQDIYHLLHCLVIPRIPLAPGMAPAVAAGLLDINAK

SEQ ID NO: 54 - DNA, 1242 bp, Escherichia coli
  source 1..1242: mol_type = genomic DNA
atgaaatggtttaacaccctaagccacaaccgttggctggaacaggaaaccgaccgcatctttgattttggtaaaaattccgtagtgccgactggttttggctggttaggcaataaagggcaaatcaaagaagagatgggcacccatctgtggatcaccgctcgtatgttgcacgtttattccgttgctgcggcgatgggtcgacctggcgcttactcgttggttgatcacggtatcaaagccatgaacggcgcactgcgtgataaaaaatatggcggctggtatgcctgcgtgaatgacgagggcgtggtggatgcctccaaacagggctatcaacacttctttgctctgctgggtgccgccagcgccgtcacaacgggtcacccggaagcgcgcaagctgctcgattacaccattgaaattatcgagaaatatttctggagcgaagaagagcagatgtgcctggaatcctgggacgaagccttcagcaaaaccgaagagtaccgcggcggcaatgccaatatgcacgcggtggaagctttcttgattgtttatgacgtcactcacgacaaaaaatggctggatcgcgcgattcgcgtggcttccgtgattatccacgacgtcgccagaaataatcattatcgcgttaacgaacacttcgatacccagtggaatccgctgccggattacaacaaagataacccggcgcatcgcttccgcgcgttcggaggtacaccaggccactggatcgaatggggccgtttaatgctgcacatccatgctgccctggaagcccgttgcgaacaaccaccagcatggctgctagaagatgccaaaggtctgtttaacgccaccgtgcgcgatgcctgggcacccgatggcgcggacgggattgtttataccgttgactgggaaggaaaaccggtggtccgcgaacgtgtacgttggcctatcgtcgaagcaatgggtacggcctacgcgctctacaccgtcactggcgatcgccagtatgaaacctggtatcaaacatggtgggagtactgcattaagtacctgatggactatgaaaatggttcctggtggcaggagctggatgcggacaataaggtcaccaccaaagtctgggacggcaaacaggatatttatcacctgctgcattgcctggtgatcccgcgtatcccgttagcgcccggcatggctccagcggttgcagcgggtctgctggatattaatgcgaaataa